European Patent Application EP 4 273 254 A1, published November 8, 2023. Title: Enzymatic method for preparing (R)-3-amino-4-aryl-butanoic acid derivatives. Applicant: Enzymicals AG Universität Greifswald. The sequence listing filed with the application follows.

SEQUENCE LISTING (2 sequences)

SEQ ID NO: 1 - protein, 442 aa, artificial sequence
  artificial sequence; sequence of transaminase of Halomonas elongata (UniProt E1V8W4)
MSHVFHRHLEQHYPTAVGGEGPYLIDAEGRRYLDACGGAAVSCLGHSDAEVIEAIREQVGRLAYAHTSFFTSEPMEALADFLIERAPSGLSSVYFVSGGSEAVEAALKMARQYFLERGEPQRKHLIARRQSYHGNTLGALATGGNTWRRRQFEPMLVEVSHVSPCYAYRDQAPGETPEAYGERLAAELEAEIERLGPETVMAFVAEPVVGATLGAVPAVPGYFKRVREICDRHGILLILDEVMCGMGRTGSLFAAEQEGVVPDLTTIAKGLGGGYQPIGATLVSERIRSAIAEGSGFFQHGHTYIGHATACAAALAVQRAIEQRDLLSRVRQLGEGLQQRLVDRFADHPHVGDIRGRGLFRGLELVAERDGKTPFDPSRKLHAEIKRTAMDEGLMCYPMGGTIDGRSGDHILLAPPFILEPYQLDEIVDKLDISLKRVFERR

SEQ ID NO: 2 - protein, 448 aa, artificial sequence
  sequence of transaminase of Halomonas elongata (UniProt E1V8W4) with His6-tag
MSHVFHRHLEQHYPTAVGGEGPYLIDAEGRRYLDACGGAAVSCLGHSDAEVIEAIREQVGRLAYAHTSFFTSEPMEALADFLIERAPSGLSSVYFVSGGSEAVEAALKMARQYFLERGEPQRKHLIARRQSYHGNTLGALATGGNTWRRRQFEPMLVEVSHVSPCYAYRDQAPGETPEAYGERLAAELEAEIERLGPETVMAFVAEPVVGATLGAVPAVPGYFKRVREICDRHGILLILDEVMCGMGRTGSLFAAEQEGVVPDLTTIAKGLGGGYQPIGATLVSERIRSAIAEGSGFFQHGHTYIGHATACAAALAVQRAIEQRDLLSRVRQLGEGLQQRLVDRFADHPHVGDIRGRGLFRGLELVAERDGKTPFDPSRKLHAEIKRTAMDEGLMCYPMGGTIDGRSGDHILLAPPFILEPYQLDEIVDKLDISLKRVFERRHHHHHH